European Patent Specification EP 3 524 672 B1, published May 28, 2025. Title: REPROGRAMMING CANCER CELLS. Applicant: MINERVA BIOTECHNOLOGIES CORPORATION BAMDAD, Cynthia. The sequence listing filed with the application follows.

SEQUENCE LISTING (6 sequences)

SEQ ID NO: 1 - protein, 45 aa, Artificial Sequence
  PSMGFR sequence
GTINVHDVETQFNQYKTEAASRYNLTISDVSVSDVPFPFSAQSGA

SEQ ID NO: 2 - DNA, 34 bp, Artificial Sequence
  primer
atcgatggatccgatggccaactgtgagcgtacc

SEQ ID NO: 3 - DNA, 33 bp, Artificial Sequence
  primer
gtggtgctcgagttcatagatccagttctgagc

SEQ ID NO: 4 - DNA, 30 bp, Artificial Sequence
  primer
gcaggaacattatacatggcggtgattctg

SEQ ID NO: 5 - DNA, 30 bp, Artificial Sequence
  primer
gccatgtataatgttcctgccaacttgtat

SEQ ID NO: 6 - protein, 35 aa, Artificial Sequence
  Truncated PSMGFR Sequence
GTINVHDVETQFNQYKTEAASRYNLTISDVSVSDV